European Patent Application EP 4 239 058 A1, published September 6, 2023. Title: Mesenchymal stem cells capable of improving tumor targeting and mass production of viruses. Applicant: Industry-Academic Cooperation Foundation, Yonsei University. The sequence listing filed with the application follows.

SEQUENCE LISTING (31 sequences)

SEQ ID NO: 1 - DNA, 1965 bp, Homo sapiens
atgaagctctccctggtggccgcgatgctgctgctgctcagcgcggcgcgggccgaggaggaggacaagaaggaggacgtgggcacggtggtcggcatcgacctggggaccacctactcctgcgtcggcgtgttcaagaacggccgcgtggagatcatcgccaacgatcagggcaaccgcatcacgccgtcctatgtcgccttcactcctgaaggggaacgtctgattggcgatgccgccaagaaccagctcacctccaaccccgagaacacggtctttgacgccaagcggctcatcggccgcacgtggaatgacccgtctgtgcagcaggacatcaagttcttgccgttcaaggtggttgaaaagaaaactaaaccatacattcaagttgatattggaggtgggcaaacaaagacatttgctcctgaagaaatttctgccatggttctcactaaaatgaaagaaaccgctgaggcttatttgggaaagaaggttacccatgcagttgttactgtaccagcctattttaatgatgcccaacgccaagcaaccaaagacgctggaactattgctggcctaaatgttatgaggatcatcaacgagcctacggcagctgctattgcttatggcctggataagagggagggggagaagaacatcctggtgtttgacctgggtggcggaaccttcgatgtgtctcttctcaccattgacaatggtgtcttcgaagttgtggccactaatggagatactcatctgggtggagaagactttgaccagcgtgtcatggaacacttcatcaaactgtacaaaaagaagacgggcaaagatgtcaggaaagacaatagagctgtgcagaaactccggcgcgaggtagaaaaggccaaacgggccctgtcttctcagcatcaagcaagaattgaaattgagtccttctatgaaggagaagacttttctgagaccctgactcgggccaaatttgaagagctcaacatggatctgttccggtctactatgaagcccgtccagaaagtgttggaagattctgatttgaagaagtctgatattgatgaaattgttcttgttggtggctcgactcgaattccaaagattcagcaactggttaaagagttcttcaatggcaaggaaccatcccgtggcataaacccagatgaagctgtagcgtatggtgctgctgtccaggctggtgtgctctctggtgatcaagatacaggtgacctggtactgcttgatgtatgtccccttacacttggtattgaaactgtgggaggtgtcatgaccaaactgattccaaggaacacagtggtgcctaccaagaagtctcagatcttttctacagcttctgataatcaaccaactgttacaatcaaggtctatgaaggtgaaagacccctgacaaaagacaatcatcttctgggtacatttgatctgactggaattcctcctgctcctcgtggggtcccacagattgaagtcacctttgagatagatgtgaatggtattcttcgagtgacagctgaagacaagggtacagggaacaaaaataagatcacaatcaccaatgaccagaatcgcctgacacctgaagaaatcgaaaggatggttaatgatgctgagaagtttgctgaggaagacaaaaagctcaaggagcgcattgatactagaaatgagttggaaagctatgcctattctctaaagaatcagattggagataaagaaaagctgggaggtaaactttcctctgaagataaggagaccatggaaaaagctgtagaagaaaagattgaatggctggaaagccaccaagatgctgacattgaagacttcaaagctaagaagaaggaactggaagaaattgttcaaccaattatcagcaaactctatggaagtgcaggccctcccccaactggtgaagaggatacagcagaaaaagatgagttgtag

SEQ ID NO: 2 - DNA, 3399 bp, Homo sapiens
atgccgcgcgctccccgctgccgagccgtgcgctccctgctgcgcagccactaccgcgaggtgctgccgctggccacgttcgtgcggcgcctggggccccagggctggcggctggtgcagcgcggggacccggcggctttccgcgcgctggtggcccagtgcctggtgtgcgtgccctgggacgcacggccgccccccgccgccccctccttccgccaggtgtcctgcctgaaggagctggtggcccgagtgctgcagaggctgtgcgagcgcggcgcgaagaacgtgctggccttcggcttcgcgctgctggacggggcccgcgggggcccccccgaggccttcaccaccagcgtgcgcagctacctgcccaacacggtgaccgacgcactgcgggggagcggggcgtgggggctgctgctgcgccgcgtgggcgacgacgtgctggttcacctgctggcacgctgcgcgctctttgtgctggtggctcccagctgcgcctaccaggtgtgcgggccgccgctgtaccagctcggcgctgccactcaggcccggcccccgccacacgctagtggaccccgaaggcgtctgggatgcgaacgggcctggaaccatagcgtcagggaggccggggtccccctgggcctgccagccccgggtgcgaggaggcgcgggggcagtgccagccgaagtctgccgttgcccaagaggcccaggcgtggcgctgcccctgagccggagcggacgcccgttgggcaggggtcctgggcccacccgggcaggacgcgtggaccgagtgaccgtggtttctgtgtggtgtcacctgccagacccgccgaagaagccacctctttggagggtgcgctctctggcacgcgccactcccacccatccgtgggccgccagcaccacgcgggccccccatccacatcgcggccaccacgtccctgggacacgccttgtcccccggtgtacgccgagaccaagcacttcctctactcctcaggcgacaaggagcagctgcggccctccttcctactcagctctctgaggcccagcctgactggcgctcggaggctcgtggagaccatctttctgggttccaggccctggatgccagggactccccgcaggttgccccgcctgccccagcgctactggcaaatgcggcccctgtttctggagctgcttgggaaccacgcgcagtgcccctacggggtgctcctcaagacgcactgcccgctgcgagctgcggtcaccccagcagccggtgtctgtgcccgggagaagccccagggctctgtggcggcccccgaggaggaggacacagacccccgtcgcctggtgcagctgctccgccagcacagcagcccctggcaggtgtacggcttcgtgcgggcctgcctgcgccggctggtgcccccaggcctctggggctccaggcacaacgaacgccgcttcctcaggaacaccaagaagttcatctccctggggaagcatgccaagctctcgctgcaggagctgacgtggaagatgagcgtgcgggactgcgcttggctgcgcaggagcccaggggttggctgtgttccggccgcagagcaccgtctgcgtgaggagatcctggccaagttcctgcactggctgatgagtgtgtacgtcgtcgagctgctcaggtctttcttttatgtcacggagaccacgtttcaaaagaacaggctctttttctaccggaagagtgtctggagcaagttgcaaagcattggaatcagacagcacttgaagagggtgcagctgcgggagctgtcggaagcagaggtcaggcagcatcgggaagccaggcccgccctgctgacgtccagactccgcttcatccccaagcctgacgggctgcggccgattgtgaacatggactacgtcgtgggagccagaacgttccgcagagaaaagagggccgagcgtctcacctcgagggtgaaggcactgttcagcgtgctcaactacgagcgggcgcggcgccccggcctcctgggcgcctctgtgctgggcctggacgatatccacagggcctggcgcaccttcgtgctgcgtgtgcgggcccaggacccgccgcctgagctgtactttgtcaaggtggatgtgacgggcgcgtacgacaccatcccccaggacaggctcacggaggtcatcgccagcatcatcaaaccccagaacacgtactgcgtgcgtcggtatgccgtggtccagaaggccgcccatgggcacgtccgcaaggccttcaagagccacgtctctaccttgacagacctccagccgtacatgcgacagttcgtggctcacctgcaggagaccagcccgctgagggatgccgtcgtcatcgagcagagctcctccctgaatgaggccagcagtggcctcttcgacgtcttcctacgcttcatgtgccaccacgccgtgcgcatcaggggcaagtcctacgtccagtgccaggggatcccgcagggctccatcctctccacgctgctctgcagcctgtgctacggcgacatggagaacaagctgtttgcggggattcggcgggacgggctgctcctgcgtttggtggatgatttcttgttggtgacacctcacctcacccacgcgaaaaccttcctcaggaccctggtccgaggtgtccctgagtatggctgcgtggtgaacttgcggaagacagtggtgaacttccctgtagaagacgaggccctgggtggcacggcttttgttcagatgccggcccacggcctattcccctggtgcggcctgctgctggatacccggaccctggaggtgcagagcgactactccagctatgcccggacctccatcagagccagtctcaccttcaaccgcggcttcaaggctgggaggaacatgcgtcgcaaactctttggggtcttgcggctgaagtgtcacagcctgtttctggatttgcaggtgaacagcctccagacggtgtgcaccaacatctacaagatcctcctgctgcaggcgtacaggtttcacgcatgtgtgctgcagctcccatttcatcagcaagtttggaagaaccccacatttttcctgcgcgtcatctctgacacggcctccctctgctactccatcctgaaagccaagaacgcagggatgtcgctgggggccaagggcgccgccggccctctgccctccgaggccgtgcagtggctgtgccaccaagcattcctgctcaagctgactcgacaccgtgtcacctacgtgccactcctggggtcactcaggacagcccagacgcagctgagtcggaagctcccggggacgacgctgactgccctggaggccgcagccaacccggcactgccctcagacttcaagaccatcctggactga

SEQ ID NO: 3 - DNA, 1491 bp, Human adenovirus type 5
atggagcgaagaaacccatctgagcggggagtacctgctggattttctggccatgcatctgtggagagcggttgtgagacacaagaatcgcctgctactgttgtcttccgtccgcccggcgataataccgacggaggagcagcagcagcagcaggaggaagccaggcggcggcggcaggagcagagcccatggaacccgagagccggcctggaccctcgggaatgaatgttgtacaggtggctgaactgtatccagaactgagacgcattttgacaattacagaggatgggcaggggctaaagggggtaaagagggagcggggggcttgtgaggctacagaggaggctaggaatctagcttttagcttaatgaccagacaccgtcctgagtgtattacttttcaacagatcaaggataattgcgctaatgagcttgatctgctggcgcagaagtattccatagagcagctgaccacttactggctgcagccaggggatgattttgaggaggctattagggtatatgcaaaggtggcacttaggccagattgcaagtacaagatcagcaaacttgtaaatatcaggaattgttgctacatttctgggaacggggccgaggtggagatagatacggaggatagggtggcctttagatgtagcatgataaatatgtggccgggggtgcttggcatggacggggtggttattatgaatgtaaggtttactggccccaattttagcggtacggttttcctggccaataccaaccttatcctacacggtgttagcttctatgggtttaacaatacctgtgtggaagcctggaccgatgtaagggttcggggctgtgccttttactgctgctggaagggggtggtgtgtcgccccaaaagcagggcttcaattaagaaatgcctctttgaaaggtgtaccttgggtatcctgtctgagggtaactccagggtgcgccacaatgtggcctccgactgtggttgcttcatgctagtgaaaagcgtggctgtgattaagcataacatggtatgtggcaactgcgaggacagggcctctcagatgctgacctgctcggacggcaactgtcacctgctgaagaccattcacgtagccagccactctcgcaaggcctggccagtgtttgagcataacatactgacccgctgttccttgcatttgggtaacaggaggggggtgttcctaccttaccaatgcaatttgagtcacactaagatattgcttgagcccgagagcatgtccaaggtgaacctgaacggggtgtttgacatgaccatgaagatctggaaggtgctgaggtacgatgagacccgcaccaggtgcagaccctgcgagtgtggcggtaaacatattaggaaccagcctgtgatgctggatgtgaccgaggagctgaggcccgatcacttggtgctggcctgcacccgcgctgagtttggctctagcgatgaagatacagattga

SEQ ID NO: 4 - DNA, 29 bp, Artificial Sequence
  BamHI/NotI forward primer
gcggatccatggagcgaagaaacccatct

SEQ ID NO: 5 - DNA, 28 bp, Artificial Sequence
  BamHI/NotI reverse primer
cggccgctcaatctgtatcttcatcgct

SEQ ID NO: 6 - DNA, 30 bp, Artificial Sequence
  HindIII forward primer
gtacaagcttatgactacgtccggcgttcc

SEQ ID NO: 7 - DNA, 30 bp, Artificial Sequence
  XbaI reverse primer
cacctctagactacatgggggtagagtcat

SEQ ID NO: 8 - DNA, 30 bp, Artificial Sequence
  CMV30
aatgtcgtaataaccccgccccgttgacgc

SEQ ID NO: 9 - DNA, 30 bp, Artificial Sequence
  XbaI sense primer
ttcatctagaatggagcgaagaaacccatc

SEQ ID NO: 10 - DNA, 30 bp, Artificial Sequence
  HindIII antisense primer
gacgaagctttcaatctgtatcttcatcgc

SEQ ID NO: 11 - DNA, 25 bp, Artificial Sequence
  hCMV forward primer
gggaggtctatataagcagagctcg

SEQ ID NO: 12 - DNA, 25 bp, Artificial Sequence
  pCA14 SV40 reverse primer
catgatcgatgctagacgatccaga

SEQ ID NO: 13 - protein, 25 aa, Artificial Sequence
  N terminus of E1B55K
MERRNPSERGVPAGFSGHASVESGC

SEQ ID NO: 14 - DNA, 40 bp, Artificial Sequence
  E1B55K In-fusion EcoRI sense primer
ccctcgtaaagaattcatggagcgaagaaacccatctgag

SEQ ID NO: 15 - DNA, 40 bp, Artificial Sequence
  E1B55K In-fusion BamHI antisense primer
gaggtggtctggatcctcaatctgtatcttcatcgctaga

SEQ ID NO: 16 - DNA, 26 bp, Artificial Sequence
  XbaI  Forward primer
gattctcgagatgaagctctccctgg

SEQ ID NO: 17 - DNA, 26 bp, Artificial Sequence
  XbaI Reverse primer
ggcctctagactacaactcatctttt

SEQ ID NO: 18 - DNA, 62 bp, Artificial Sequence
  pLNCX neo Top strand
agcttcacgtgccagcacagtggcggccgctcgagtcgacgggcccgtttaaacgttaacat

SEQ ID NO: 19 - DNA, 60 bp, Artificial Sequence
  pLNCX neo Bottom strand
cgatgttaacgtttaaacgggcccgtcgactcgagcggccgccactgtgctggcacgtga

SEQ ID NO: 20 - DNA, 20 bp, Artificial Sequence
  E4 ORF Forward primer
cgtggtcaaactctacagcc

SEQ ID NO: 21 - DNA, 20 bp, Artificial Sequence
  E4 ORF Reverse primer
gcatgagcatgactacgatg

SEQ ID NO: 22 - DNA, 912 bp, Artificial Sequence
  Flag-E4orf6
gactacaaagacgatgacgacaagcttatgactacgtccggcgttccatttggcatgacactacgaccaacacgatctcggttgtctcggcgcactccgtacagtagggatcgtctacctccttttgagacagaaacccgcgctaccatactggaggatcatccgctgctgcccgaatgtaacactttgacaatgcacaacgtgagttacgtgcgaggtcttccctgcagtgtgggatttacgctgattcaggaatgggttgttccctgggatatggttctaacgcgggaggagcttgtaatcctgaggaagtgtatgcacgtgtgcctgtgttgtgccaacattgatatcatgacgagcatgatgatccatggttacgagtcctgggctctccactgtcattgttccagtcccggttccctgcagtgtatagccggcgggcaggttttggccagctggtttaggatggtggtggatggcgccatgtttaatcagaggtttatatggtaccgggaggtggtgaattacaacatgccaaaagaggtaatgtttatgtccagcgtgtttatgaggggtcgccacttaatctacctgcgcttgtggtatgatggccacgtgggttctgtggtccccgccatgagctttggatacagcgccttgcactgtgggattttgaacaatattgtggtgctgtgctgcagttactgtgctgatttaagtgagatcagggtgcgctgctgtgcccggaggacaaggcgccttatgctgcgggcggtgcgaatcatcgctgaggagaccactgccatgttgtattcctgcaggacggagcggcggcggcagcagtttattcgcgcgctgctgcagcaccaccgccctatcctgatgcacgattatgactctacccccatgtag

SEQ ID NO: 23 - DNA, 1196 bp, Artificial Sequence
  sample 2-Fig. 7
aaccgtcagaattgatctaccatggactacaaagacgatgacgacaagcttatgactacgtccggcgttccatttggcatgacactacgaccaacacgatctcggttgtctcggcgcactccgtacagtagggatcgtctacctccttttgagacagaaacccgcgctaccatactggaggatcatccgctgctgcccgaatgtaacactttgacaatgcacaacgtgagttacgtgcgaggtcttccctgcagtgtgggatttacgctgattcaggaatgggttgttccctgggatatggttctaacgcgggaggagcttgtaatcctgaggaagtgtatgcacgtgtgcctgtgttgtgccaacattgatatcatgacgagcatgatgatccatggttacgagtcctgggctctccactgtcattgttccagtcccggttccctgcagtgtatagccggcgggcaggttttggccagctggtttaggatggtggtggatggcgccatgtttaatcagaggtttatatggtaccgggaggtggtgaattacaacatgccaaaagaggtaatgtttatgtccagcgtgtttatgaggggtcgccacttaatctacctgcgcttgtggtatgatggccacgtgggttctgtggtccccgccatgagctttggatacagcgccttgcactgtgggattttgaacaatattgtggtgctgtgctgcagttactgtgctgatttaagtgagatcagggtgcgctgctgtgcccggaggacaaggcgccttatgctgcgggcggtgcgaatcatcgctgaggagaccactgccatgttgtattcctgcaggacggagcggcggcggcagcagtttattcgcgcgctgctgcagcaccaccgccctatcctgatgcacgattatgactctacccccatgtagtctagaggatcccgggtggcatccctgtgacccctccccagtgcctctcctggccctggaagttgccactccagtgcccaccagccttgtcctaataaaattaagttgcatcattttgtctgactaggtgtccttctataatattatggggtggagggggggggtatggaaccaaggggcaagttgggaaaaaaacctgaagggcctgcgggtcttattgggaaccaaactgggagtgcagtggaccaattttgggttcc

SEQ ID NO: 24 - DNA, 960 bp, Artificial Sequence
  pCA14-E1B55K forward
aagacaccgggaccgatccagcctggggatcttcgagtcgagggatccctcgagtctagaatggagcgaagaaacccatctgagcggggagtacctgctggattttctggccatgcatctgtggagagcggttgtgagacacaagaatcgcctgctactgttgtcttccgtccgcccggcgataataccgacggaggagcagcagcagcagcaggaggaagccaggcggcggcggcaggagcagagcccatggaacccgagagccggcctggaccctcgggaatgaatgttgtacaggtggctgaactgtatccagaactgagacgcattttgacaattacagaggatgggcaggggctaaagggggtaaagagggagcggggggcttgtgaggctacagaggaggctaggaatctagcttttagcttaatgaccagacaccgtcctgagtgtattacttttcaacagatcaaggataattgcgctaatgagcttgatctgctggcgcagaagtattccatagagcagctgaccacttactggctgcagccaggggatgattttgaggaggctattagggtatatgcaaaggtggcacttaggccagattgcaagtacaagatcagcaaacttgtaaatatcaggaattgttgctacatttctgggaacggggccgaggtggagatagatacggaggatagggtggcctttagatgtagcatgataaatatgtggccgggggtgcttggcatggacggggtggttattatgaatgtaaggtttactggccccaattttagcggtacggttttcctggccaataccaaccttatcctacacggtgttagcttctatgggtttaacaatacctgtgtggaagcctggaccgatgtaagggttcggggctgtgccttttactgctgctggaagggggtggtgtgtcgccccaaaagcagggct

SEQ ID NO: 25 - DNA, 1017 bp, Artificial Sequence
  pCA14-E1B55K-reverse
tttggtccaaccggggatgatttgagggggcttttgggtttttgcaaaggtgcccttaggccagattgcaattacaaaatcagcaaacttgtaaatttcaggaattgttgctacatttctgggaacggggccgaggtggagatagatacggaggatagggtggcctttagatgtagcatgataaatatgtggccgggggtgcttggcatggacggggtggttattatgaatgtaaggtttactggccccaattttagcggtacggttttcctggccaataccaaccttatcctacacggtgttagcttctatgggtttaacaatacctgtgtggaagcctggaccgatgtaagggttcggggctgtgccttttactgctgctggaagggggtggtgtgtcgccccaaaagcagggcttcaattaagaaatgcctctttgaaaggtgtaccttgggtatcctgtctgagggtaactccagggtgcgccacaatgtggcctccgactgtggttgcttcatgctagtgaaaagcgtggctgtgattaagcataacatggtatgtggcaactgcgaggacagggcctctcagatgctgacctgctcggacggcaactgtcacctgctgaagaccattcacgtagccagccactctcgcaaggcctggccagtgtttgagcataacatactgacccgctgttccttgcatttgggtaacaggaggggggtgttcctaccttaccaatgcaatttgagtcacactaagatattgcttgagcccgagagcatgtccaaggtgaacctgaacggggtgtttgacatgaccatgaagatctggaaggtgctgaggtacgatgagacccgcaccaggtgcagaccctgcgagtgtggcggtaaacatattaggaaccagcctgtgatgctggatgtgaccgaggagctgaggcccgatcacttggtgctggcctgcacccgcgctgagtttggctctagcgatgaagatacagattgaaagcttgtc

SEQ ID NO: 26 - DNA, 1172 bp, Artificial Sequence
  primer E1B55K In-fusion EcoRI sense
ccggggggcagtacctgctggattctctggccatgcatctgtggagagcggttgtgagacacaagaatcgcctgctactgttgtcttccgtccgcccggcgataataccgacggaggagcagcagcagcagcaggaggaagccaggcggcggcggcaggagcagagcccatggaacccgagagccggcctggaccctcgggaatgaatgttgtacaggtggctgaactgtatccagaactgagacgcattttgacaattacagaggatgggcaggggctaaagggggtaaagagggagcggggggcttgtgaggctacagaggaggctaggaatctagcttttagcttaatgaccagacaccgtcctgagtgtattacttttcaacagatcaaggataattgcgctaatgagcttgatctgctggcgcagaagtattccatagagcagctgaccacttactggctgcagccaggggatgattttgaggaggctattagggtatatgcaaaggtggcacttaggccagattgcaagtacaagatcagcaaacttgtaaatatcaggaattgttgctacatctctgggaacggggccgaggtggagatagatacggaggatagggtggcctttagatgtagcatgataaatatgtggccgggggtgcttggcatggacggggtggttattatgaatgtaaggtttactggccccaattttagcggtacggttttcctggccaataccaaccttatcctacacggtgttagcttctatgggtttaacaatacctgtgtggaagcctggaccgatgtaagggttcggggctgtgccttttactgctgctggaagggggtggtgtgtcgccccaaaagcagggcttcaattaagaaatgcctctttgaaaggtgtaccttgggtatcctgtctgagggtaactccagggtgcgccacaatgtggcctccgactgtggttgcttcatgctagtgaaaagcgtggctgtgattaagcataacatggtatgtggcaactgcgaggacagggcctctcagatgctgacctgctcggacggcaactgtcacctgctgaagacattcacgtagccagccctttcgcaaggctggccagggttgagcatacctactgaccccctgttccttgctttgggaaaaa

SEQ ID NO: 27 - DNA, 686 bp, Artificial Sequence
  primer: E1B55K internal primer
acctgtaatttgtttatttgggcgtaggtcgggcgtgcttttactgctgctggaagggggtggtgtgtcgccccaaaagcagggcttcaattaagaaatgcctctttgaaaggtgtaccttgggtatcctgtctgagggtaactccagggtgcgccacaatgtggcctccgactgtggttgcttcatgctagtgaaaagcgtggctgtgattaagcataacatggtatgtggcaactgcgaggacagggcctctcagatgctgacctgctcggacggcaactgtcacctgctgaagaccattcacgtagccagccactctcgcaaggcctggccagtgtttgagcataacatactgacccgctgttccttgcatttgggtaacaggaggggggtgttcctaccttaccaatgcaatttgagtcacactaagatattgcttgagcccgagagcatgtccaaggtgaacctgaacggggtgtttgacatgaccatgaagatctggaaggtgctgaggtacgatgagacccgcaccaggtgcagaccctgcgagtgtggcggtaaacatattaggaaccagcctgtgatgctggatgtgaccgaggagctgaggcccgatcacttggtgctggcctgcacccgcgctgagtttggctctagcgatgaagatacagattgaggatccaga

SEQ ID NO: 28 - DNA, 483 bp, Artificial Sequence
  E1B55K 5' near internal reverse primer
aaagaattcatggagcgaagaaacccatctgagcggggagtacctgctggattctctggccatgcatctgtggagagcggttgtgagacacaagaatcgcctgctactgttgtcttccgtccgcccggcgataataccgacggaggagcagcagcagcagcaggaggaagccaggcggcggcggcaggagcagagcccatggaacccgagagccggcctggaccctcgggaatgaatgttgtacaggtggctgaactgtatccagaactgagacgcattttgacaattacagaggatgggcaggggctaaagggggtaaagagggagcggggggcttgtgaggctacagaggaggctaggaatctagcttttagcttaatgaccagacaccgtcctgagtgtattacttttcaacagatcaaggataattgcgctaatgagctgatctgcgcgcagacgcgccaacaaaacaagagtccagtc

SEQ ID NO: 29 - DNA, 1246 bp, Artificial Sequence
  primer:E1B55K In-fusion BamHI antisense
aaaggatggcagggctaaaggggtaaagaggagcgggggcttggaggctacagaggaggctaggaatctagcttttagcttaatgaccagacaccgtcctgagtgtattacttttcaacagatcaaggataattgcgctaatgagcttgatctgctggcgcagaagtattccatagagcagctgaccacttactggctgcagccaggggatgattttgaggaggctattagggtatatgcaaaggtggcacttaggccagattgcaagtacaagatcagcaaacttgtaaatatcaggaattgttgctacatctctgggaacggggccgaggtggagatagatacggaggatagggtggcctttagatgtagctctgggaacggggccgaggtggagatagatacggaggatagggtggcctttagatgtagctctgggaacggggccgaggtggagatagatacggaggatagggtggcctttagatgtagctttactggccccaattttagcggtacggttttcctggccaataccaaccttatcctacacggtgttagcttctatgggtttaacaatacctgtgtggaagcctggaccgatgtaagggttcggggctgtgccttttactgctgctggaagggggtggtgtgtcgccccaaaagcagggcttcaattaagaaatgcctctttgaaaggtgtaccttgggtatcctgtctgagggtaactccagggtgcgccacaatgtggcctccgactgtggttgcttcatgctagtgaaaagcgtggctgtgattaagcataacatggtatgtggcaactgcgaggacagggcctctcagatgctgacctgctcggacggcaactgtcacctgctgaagaccattcacgtagccagccactctcgcaaggcctggccagtgtttgagcataacatactgacccgctgttccttgcatttgggtaacaggaggggggtgttcctaccttaccaatgcaatttgagtcacactaagatattgcttgagcccgagagcatgtccaaggtgaacctgaacggggtgtttgacatgaccatgaagatctggaaggtgctgaggtacgatgagacccgcaccaggtgcagaccctgcgagtgtggcggtaaacatattaggaaccagcctgtgatgctggatgtgaccgaggagctgaggcccgatcacttggtgctggcctgcacccgcgctgagtttggcccccgt

SEQ ID NO: 30 - DNA, 995 bp, Artificial Sequence
  pcDNA3.1 GRP78 forward
tggtggaattctgcagatatccagcacagtggcggccgctcgagatgaagctctccctggtggccgcgatgctgctgctgctcagcgcggcgcgggccgaggaggaggacaagaaggaggacgtgggcacggtggtcggcatcgacctggggaccacctactcctgcgtcggcgtgttcaagaacggccgcgtggagatcatcgccaacgatcagggcaaccgcatcacgccgtcctatgtcgccttcactcctgaaggggaacgtctgattggcgatgccgccaagaaccagctcacctccaaccccgagaacacggtctttgacgccaagcggctcatcggccgcacgtggaatgacccgtctgtgcagcaggacatcaagttcttgccgttcaaggtggttgaaaagaaaactaaaccatacattcaagttgatattggaggtgggcaaacaaagacatttgctcctgaagaaatttctgccatggttctcactaaaatgaaagaaaccgctgaggcttatttgggaaagaaggttacccatgcagttgttactgtaccagcctattttaatgatgcccaacgccaagcaaccaaagacgctggaactattgctggcctaaatgttatgaggatcatcaacgagcctacggcagctgctattgcttatggcctggataagagggagggggagaagaacatcctggtgtttgacctgggtggcggaaccttcgatgtgtctcttctcaccattgacaatggtgtcttcgaagttgtggccactaatggagatactcatctgggtggagaagactttgaccagcgtgtcatggaacacttcatcaaactgtacaaaaagaagacgggcaaagatgtcaggaaagacaatagagctgtgcagaaactccggcgcgaggtagaaaaggccaaacgggccctgtcttctcagcatcaagcaagaattgaaattgagtccttctatgaaggagaagac

SEQ ID NO: 31 - DNA, 1046 bp, Artificial Sequence
  pcDNA3.1 GRP78 reverse
tctatgaaggagaagacttttctgagaccctgactcgggccaaatttgaagagctcaacatggatctgttccggtctactatgaagcccgtccagaaagtgttggaagattctgatttgaagaagtctgatattgatgaaattgttcttgttggtggctcgactcgaattccaaagattcagcaactggttaaagagttcttcaatggcaaggaaccatcccgtggcataaacccagatgaagctgtagcgtatggtgctgctgtccaggctggtgtgctctctggtgatcaagatacaggtgacctggtactgcttgatgtatgtccccttacacttggtattgaaactgtgggaggtgtcatgaccaaactgattccaaggaacacagtggtgcctaccaagaagtctcagatcttttctacagcttctgataatcaaccaactgttacaatcaaggtctatgaaggtgaaagacccctgacaaaagacaatcatcttctgggtacatttgatctgactggaattcctcctgctcctcgtggggtcccacagattgaagtcacctttgagatagatgtgaatggtattcttcgagtgacagctgaagacaagggtacagggaacaaaaataagatcacaatcaccaatgaccagaatcgcctgacacctgaagaaatcgaaaggatggttaatgatgctgagaagtttgctgaggaagacaaaaagctcaaggagcgcattgatactagaaatgagttggaaagctatgcctattctctaaagaatcagattggagataaagaaaagctgggaggtaaactttcctctgaagataaggagaccatggaaaaagctgtagaagaaaagattgaatggctggaaagccaccaagatgctgacattgaagacttcaaagctaagaagaaggaactggaagaaattgttcaaccaattatcagcaaactctatggaagtgcaggccctcccccaactggtgaagaggatacagcagaaaaagatgagttgtagtctagagtcccgtaa